European Patent Application EP 4 407 315 A1, published July 31, 2024. Title: DIAGNOSIS AND TREATMENT OF NEUROGENIC HETEROTOPIC OSSIFICATION. Applicant: SERVIZO GALEGO DE SAÚDE. The sequence listing filed with the application follows.

SEQUENCE LISTING (6 sequences)

SEQ ID NO: 1 - RNA, 25 nt, synthetic construct
  source 1..25: mol_type = other RNA
  modified_base 24: mod_base = OTHER; note = Thymine
gtggcaaatcaacagtcatcagcta

SEQ ID NO: 2 - RNA, 27 nt, synthetic construct
  source 1..27: mol_type = other RNA
tagctgatgactgttgatttgccacag

SEQ ID NO: 3 - RNA, 25 nt, synthetic construct
  source 1..25: mol_type = other RNA
  modified_base 24: mod_base = OTHER; note = Thymine
  modified_base 25: mod_base = OTHER; note = Thymine
gttttcaaaaccaagtatcacactt

SEQ ID NO: 4 - RNA, 27 nt, synthetic construct
  source 1..27: mol_type = other RNA
aagtgtgatacttggttttgaaaacat

SEQ ID NO: 5 - RNA, 25 nt, synthetic construct
  source 1..25: mol_type = other RNA
ctacattgatgagctactcatccca

SEQ ID NO: 6 - RNA, 27 nt, synthetic construct
  source 1..27: mol_type = other RNA
tgggatgagtagctcatcaatgtagtg